European Patent Application EP 4 764 497 A1, published June 24, 2026. Title: HERV ENV DETECTION TEST. Applicant: GENEURO SA. Application EP. The sequence listing filed with the application follows.

SEQUENCE LISTING (22 sequences)

SEQ ID NO: 1 - protein, 10 aa, synthetic construct
SASSSVSYMY

SEQ ID NO: 2 - protein, 7 aa, synthetic construct
RTSNLAS

SEQ ID NO: 3 - protein, 9 aa, synthetic construct
QQYQSLPLT

SEQ ID NO: 4 - protein, 5 aa, synthetic construct
DYEMH

SEQ ID NO: 5 - protein, 17 aa, synthetic construct
AVAPETGGTAYNQKFKG

SEQ ID NO: 6 - protein, 7 aa, synthetic construct
TVVPFAY

SEQ ID NO: 7 - protein, 106 aa, synthetic construct
QIQLTQSPSSLSASVGDRVTITCSASSSVSYMYWYQQKPGKAPKAWIYRTSNLASGVPSRFSGSGSGTDYTLTISSLQPEDFATYYCQQYQSLPLTFGGGTKVEIK

SEQ ID NO: 8 - protein, 116 aa, synthetic construct
QVQLVQSGAEVKKPGSSVKVSCKASGYTFTDYEMHWVRQAPGQGLEWIGAVAPETGGTAYNQKFKGRATITADKSTSTAYMELSSLRSEDTAVYYCTSTVVPFAYWGQGTLVTVSS

SEQ ID NO: 9 - protein, 11 aa, synthetic construct
QSLLDSDGKTY

SEQ ID NO: 10 - skipped

SEQ ID NO: 11 - protein, 9 aa, synthetic construct
LQATHFPWT

SEQ ID NO: 12 - protein, 8 aa, synthetic construct
GYTFTSYW

SEQ ID NO: 13 - protein, 8 aa, synthetic construct
IDPYDSET

SEQ ID NO: 14 - protein, 10 aa, synthetic construct
ASLYYYGISL

SEQ ID NO: 15 - DNA, 1647 bp, synthetic construct
  source 1..1647: mol_type = other DNA
atggccctcccttatcatacttttctctttactgttctcttaccccctttcgctctcactgcaccccctccatgctgctgtacaaccagtagctccccttaccaagagtttctatggagaacgcggcttcctggaaatattgatgccccatcatataggagtttatctaagggaaactccaccttcactgcccacacccatatgccccgcaactgctataactctgccactctttgcatgcatgcaaatactcattattggacagggaaaatgattaatcctagttgtcctggaggacttggagccactgtctgttggacttacttcacccataccagtatgtctgatgggggtggaattcaaggtcaggcaagagaaaaacaagtaaaggaagcaatctcccaactgacccggggacatagcacccctagcccctacaaaggactagttctctcaaaactacatgaaaccctccgtacccatactcgcctggtgagcctatttaataccaccctcactcggctccatgaggtctcagcccaaaaccctactaactgttggatgtgcctccccctgcacttcaggccatacatttcaatccctgttcctgaacaatggaacaacttcagcacagaaataaacaccacttccgttttagtaggacctcttgtttccaatctggaaataacccatacctcaaacctcacctgtgtaaaatttagcaatactatagacacaaccagctcccaatgcatcaggtgggtaacacctcccacacgaatagtctgcctaccctcaggaatattttttgtctgtggtacctcagcctatcattgtttgaatggctcttcagaatctatgtgcttcctctcattcttagtgccccctatgaccatctacactgaacaagatttatacaatcatgtcgtacctaagccccacaacaaaagagtacccattcttccttttgttatcagagcaggagtgctaggcagactaggtactggcattggcagtatcacaacctctactcagttctactacaaactatctcaagaaataaatggtgacatggaacaggtcactgactccctggtcaccttgcaagatcaacttaactccctagcagcagtagtccttcaaaatcgaagagctttagacttgctaaccgccaaaagagggggaacctgtttatttttaggagaagaacgctgttattatgttaatcaatccagaattgtcactgagaaagttaaagaaattcgagatcgaatacaatgtagagcagaggagcttcaaaacaccgaacgctggggcctcctcagccaatggatgccctggactctccccttcttaggacctctagcagctataatatttttactcctctttggaccctgtatcttcaacttccttgttaagtttgtctcttccagaattgaagctgtaaagctacaaatagttcttcaaatggaaccccagatgcagtccatgactaaaatctaccgtggacccctggaccggcctgctagactatgctctgatgttaatgacattgaagtcacccctcccgaggaaatctcaactgcacaacccctactacactccaattcagtaggaagcagtcatcatcatcatcatcattag

SEQ ID NO: 16 - protein, 548 aa, synthetic construct
MALPYHTFLFTVLLPPFALTAPPPCCCTTSSSPYQEFLWRTRLPGNIDAPSYRSLSKGNSTFTAHTHMPRNCYNSATLCMHANTHYWTGKMINPSCPGGLGATVCWTYFTHTSMSDGGGIQGQAREKQVKEAISQLTRGHSTPSPYKGLVLSKLHETLRTHTRLVSLFNTTLTRLHEVSAQNPTNCWMCLPLHFRPYISIPVPEQWNNFSTEINTTSVLVGPLVSNLEITHTSNLTCVKFSNTIDTTSSQCIRWVTPPTRIVCLPSGIFFVCGTSAYHCLNGSSESMCFLSFLVPPMTIYTEQDLYNHVVPKPHNKRVPILPFVIRAGVLGRLGTGIGSITTSTQFYYKLSQEINGDMEQVTDSLVTLQDQLNSLAAVVLQNRRALDLLTAKRGGTCLFLGEERCYYVNQSRIVTEKVKEIRDRIQCRAEELQNTERWGLLSQWMPWTLPFLGPLAAIIFLLLFGPCIFNFLVKFVSSRIEAVKLQIVLQMEPQMQSMTKIYRGPLDRPARLCSDVNDIEVTPPEEISTAQPLLHSNSVGSSHHHHHH

SEQ ID NO: 17 - DNA, 1653 bp, synthetic construct
  source 1..1653: mol_type = other DNA
atgcatcatcatcatcatcatctgccgatgccggccggtgcagcagcagcaaattatacctattgggcctatgttccgtttccgccgctgattcgcgccgtgacctggatggataatccgaccgaagtgtatgtgaatgatagcgtgtgggttccgggtccgattgatgatcgttgcccggcaaaaccggaagaagaaggcatgatgattaatattagcattggctatcactacccgccgatttgcctgggtcgtgccccgggttgcctgatgccggctgttcagaattggctggtggaagtgccgaccgtgagtccgatttgtcgttttacctatcatatggttagcggtatgagtctgcgcccgcgcgttaattatctgcaggattttagttatcagcgcagcctgaaatttcgcccgaaaggtaaaccgtgtccgaaagaaattccgaaagaaagtaaaaataccgaagttctggtgtgggaagaatgtgtggcaaatagtgccgttattctgcagaataatgaatttggcaccattattgattgggcaccgcgtggtcagttttatcataattgcagtggtcagacccagagttgcccgagtgcacaggtgagtccggccgtggatagtgatctgaccgaaagcctggataaacataaacataaaaagctgcagagcttttatccgtgggaatggggtgaaaaaggtattagcaccccgcgtccgaaaattgttagtccggtgagcggcccggaacatccggaactgtggcgcctgaccgttgcaagtcatcatattcgcatttggagcggcaatcagaccctggaaacccgcgatcgcaaaccgttttataccattgatctgaatagtagtctgaccgtgccgctgcagagttgcgtgaaaccgccgtatatgctggtggttggcaatattgttattaagccggatagccagaccattacctgtgaaaattgtcgcctgctgacctgtattgatagcacctttaattggcagcatcgcattctgctggttcgcgcccgtgaaggcgtttggattccggttagtatggatcgtccgtgggaagcaagcccgagcgttcatattctgaccgaagtgctgaaaggcgtgctgaatcgtagcaaacgttttatttttaccctgattgcagtgattatgggtctgattgcagttaccgcaaccgcagcagttgccggcgttgcactgcatagtagcgttcagagcgttaattttgttaatgattggcagaaaaacagcacccgtctgtggaatagccagagcagtattgatcagaaactggcaaatcagattaatgatctgcgccagaccgttatttggatgggtgaccgtctgatgagtctggaacatcgctttcagctgcagtgtgattggaataccagcgatttttgtattaccccgcagatctataatgaaagcgaacatcattgggatatggttcgccgccatctgcagggccgtgaagataatctgaccctggatattagcaaactgaaagaacagattttcgaagccagtaaagcccatctgaatctggttccgggtaccgaagccattgccggtgtggccgatggtctggccaatctgaatccggttacctgggtgaaaacctaa

SEQ ID NO: 18 - protein, 550 aa, synthetic construct
MHHHHHHLPMPAGAAAANYTYWAYVPFPPLIRAVTWMDNPTEVYVNDSVWVPGPIDDRCPAKPEEEGMMINISIGYHYPPICLGRAPGCLMPAVQNWLVEVPTVSPICRFTYHMVSGMSLRPRVNYLQDFSYQRSLKFRPKGKPCPKEIPKESKNTEVLVWEECVANSAVILQNNEFGTIIDWAPRGQFYHNCSGQTQSCPSAQVSPAVDSDLTESLDKHKHKKLQSFYPWEWGEKGISTPRPKIVSPVSGPEHPELWRLTVASHHIRIWSGNQTLETRDRKPFYTIDLNSSLTVPLQSCVKPPYMLVVGNIVIKPDSQTITCENCRLLTCIDSTFNWQHRILLVRAREGVWIPVSMDRPWEASPSVHILTEVLKGVLNRSKRFIFTLIAVIMGLIAVTATAAVAGVALHSSVQSVNFVNDWQKNSTRLWNSQSSIDQKLANQINDLRQTVIWMGDRLMSLEHRFQLQCDWNTSDFCITPQIYNESEHHWDMVRRHLQGREDNLTLDISKLKEQIFEASKAHLNLVPGTEAIAGVADGLANLNPVTWVKT

SEQ ID NO: 19 - DNA, 2100 bp, synthetic construct
  source 1..2100: mol_type = other DNA
atgaacccatcggagatgcaaagaaaagcacctccgcggagacggagacaccgcaatcgagcaccgttgactcacaagatgaacaaaatggtgacgtcagaagaacagatgaagttgccatccaccaagaaggcagagccgccgacttgggcacaactaaagaagctgacgcagttagctacaaaatatctagagaacacaaaggtgacacaaaccccagagagtatgctgcttgcagccttgatgattgtatcaatggtggtaagtctccctatgcctgcaggagcagctgcagctaactatacctactgggcctatgtgcctttcccgcccttaattcgggcagtcacatggatggataatcctatagaaatatatgttaatgatagtgtatgggtacctggccccacagatgattgctgccctgccaaacctgaggaagaagggatgatgataaatatttccattgggtatcgttatcctcctatttgcctagggagagcaccaggatgtttaatgcctgcagtccaaaattggttggtagaagtacctactgtcagtcccatcagtagattcacttatcacatggtaagcgggatgtcactcaggccacgggtaaattatttacaagacttttcttatcaaagatcattaaaatttagacctaaagggaaaccttgccccaaggaaattcccaaagaatcaaaaaatacagaagttttagtttgggaagaatgtgtggccaatagtgcggtgatattacaaaacaatgaattcggaactcttatagattgggcacctcgaggtcaattctaccacaattgctcaggacaaactcagtcgtgtccaagtgcacaagtgagtccagctgttgatagcgacttaacagaaagtttagacaaacataagcataaaaaattgcagtctttctacccttgggaatggggagaaaaaggaatctctaccgcaagaccaaaaataataagtcctgtttctggtcctgaacatccagaattatggaggcttactgtggcctcacaccacattagaatttggtctggaaatcaaactttagaaacaagagatcgtaagccattttatactatcgacctaaattccagtctaacagttcctttacaaagttgcgtaaagcccccttatatgctagttgtaggaaatatagttattaaaccagactcccagactataacctgtgaaaattgtagattgcttacttgcattgattcaacttttaattggcaacaccgtattctgctggtgagagcaagagagggcgtgtggattcctgtgtccatggaccgaccgtgggaggcctcaccatccgtccatattttgactgaagtattaaaaggtgttttaaatagatccaaaagattcatttttactttaattgcagtgattatgggattaattgcagtcacagctacggctgctgtagcaggagttgcattgcactcttctgttcagtcagtaaactttgttaatgattggcaaaataattctacaagattgtggaattcacaatctagtattgatcaaaaattggcaaatcaaattaatgatcttagacaaactgtcatttggatgggagacaggctcatgagcttagaacatcgtttccagttacaatgtgactggaatacgtcagatttttgtattacaccccaaatttataatgagtctgagcatcactgggacatggttagatgccatctacagggaagagaagataatctcactttagacatttccaaattaaaagaacaaatttttgaagcatcaaaagcccatttaaatttggtgccaggaactgaggcaattgcaggagttgctgatggcctcgcaaatcttaacactgtcacttgggttaagaccattggaagtactacaattataaatctcatattaatccttgtgtgcctgttttgtctgttgttagtctacaggtgtacccaacagctccgacgagacagcgaccatcgagaacgggccatgatgacgatggtggttttgtcgaaaagaaaagggggaaatgtggggaaaagcaagagagatcagattgttactgtgtctgtgtag

SEQ ID NO: 20 - protein, 699 aa, synthetic construct
MNPSEMQRKAPPRRRRHRNRAPLTHKMNKMVTSEEQMKLPSTKKAEPPTWAQLKKLTQLATKYLENTKVTQTPESMLLAALMIVSMVVSLPMPAGAAAANYTYWAYVPFPPLIRAVTWMDNPIEIYVNDSVWVPGPTDDCCPAKPEEEGMMINISIGYRYPPICLGRAPGCLMPAVQNWLVEVPTVSPISRFTYHMVSGMSLRPRVNYLQDFSYQRSLKFRPKGKPCPKEIPKESKNTEVLVWEECVANSAVILQNNEFGTLIDWAPRGQFYHNCSGQTQSCPSAQVSPAVDSDLTESLDKHKHKKLQSFYPWEWGEKGISTARPKIISPVSGPEHPELWRLTVASHHIRIWSGNQTLETRDRKPFYTIDLNSSLTVPLQSCVKPPYMLVVGNIVIKPDSQTITCENCRLLTCIDSTFNWQHRILLVRAREGVWIPVSMDRPWEASPSVHILTEVLKGVLNRSKRFIFTLIAVIMGLIAVTATAAVAGVALHSSVQSVNFVNDWQNNSTRLWNSQSSIDQKLANQINDLRQTVIWMGDRLMSLEHRFQLQCDWNTSDFCITPQIYNESEHHWDMVRCHLQGREDNLTLDISKLKEQIFEASKAHLNLVPGTEAIAGVADGLANLNTVTWVKTIGSTTIINLILILVCLFCLLLVYRCTQQLRRDSDHRERAMMTMVVLSKRKGGNVGKSKRDQIVTVSV

SEQ ID NO: 21 - DNA, 1545 bp, synthetic construct
  source 1..1545: mol_type = other DNA
catatgaatccgtctgaaatgcaacgtaaagctccgccacgtcgtcgtcgtcaccgtaatcgtgctccgctgacccacaaaatgaataaaatggttacctctgaagaacagatgaaactgccgtctaccaaaaaagcggaaccgccgacctgggcgcagctgaagaaactgactcagctggctaccaaatatctggaaaatactaaagtaacccagactccagaatccatgctgctggctgcactgatgattgtttccatggtagtttccctgccgatgccagctggtgcggcagctgccaattacacctactgggcatacgtgccgttcccgccgctgattcgtgcagtgacctggatggataatccgattgaaatctatgtaaatgattctgtttgggtaccgggtccgactgatgactgctgcccggccaaaccggaagaagaaggcatgatgattaatatcagcatcggttaccgctatccgccaatctgcctgggtcgtgcaccgggttgcctgatgccggcggttcagaattggctggttgaagtgccgaccgtaagcccgatttctcgttttacctaccacatggtttctggcatgtccctgcgtccgcgtgtgaattacctgcaagacttcagctaccagcgttctctgaaattccgcccgaagggcaaaccgtgtccgaaggaaatcccgaaggaaagcaagaataccgaagtgctggtttgggaagagtgtgtagcgaatagcgctgtgatcctgcagaataatgagtttggtaccctgattgactgggctccgcgtggtcagttctaccacaattgcagcggtcagacccagtcttgtccgtctgcacaggtttctccggcggttgattctgacctgaccgaaagcctggacaaacacaaacacaagaaactgcagtctttctatccgtgggaatggggcgaaaaaggcatcagcactgcccgcccaaaaatcatctctccagttagcggtccggagcatccagagctgtggcgtctgactgttgcctctcaccacatccgcatctggtccggtaatcagactctggagactcgtgaccgcaaaccattctacaccattgacctgaattccagcctgactgttccgctgcagtcttgcgtgaaaccgccgtacatgctggtagtaggcaatatcgtaatcaaaccagattcccagaccatcacctgcgagaattgccgcctgctgacttgcattgactccaccttcaattggcagcaccgcatcctgctggtgcgtgcgcgcgaaggcgtgtggattccggtttccatggatcgtccgtgggaagcgtctccgtctgtgcacatcctgactgaagtgctgaaaggcgttctgaatcgctccaaacgccaaaaaatccatttttacttcaattgttccgactatggcatcaattgcagccacagctacggttgttgttcccgttcctgcatcgcgctgttctgcagcgtttccaaactgtgtggttccagccatcatcaccaccaccattaataa

SEQ ID NO: 22 - protein, 512 aa, synthetic construct
MNPSEMQRKAPPRRRRHRNRAPLTHKMNKMVTSEEQMKLPSTKKAEPPTWAQLKKLTQLATKYLENTKVTQTPESMLLAALMIVSMVVSLPMPAGAAAANYTYWAYVPFPPLIRAVTWMDNPIEIYVNDSVWVPGPTDDCCPAKPEEEGMMINISIGYRYPPICLGRAPGCLMPAVQNWLVEVPTVSPISRFTYHMVSGMSLRPRVNYLQDFSYQRSLKFRPKGKPCPKEIPKESKNTEVLVWEECVANSAVILQNNEFGTLIDWAPRGQFYHNCSGQTQSCPSAQVSPAVDSDLTESLDKHKHKKLQSFYPWEWGEKGISTARPKIISPVSGPEHPELWRLTVASHHIRIWSGNQTLETRDRKPFYTIDLNSSLTVPLQSCVKPPYMLVVGNIVIKPDSQTITCENCRLLTCIDSTFNWQHRILLVRAREGVWIPVSMDRPWEASPSVHILTEVLKGVLNRSKRQKIHFYFNCSDYGINCSHSYGCCSRSCIALFCSVSKLCGSSHHHHHH